European Patent Application EP 4 707 297 A1, published March 11, 2026. Title: 면역글로불린 Fc 영역 또는 이의 변이체를 포함하는 재조합 세포외 소포체 및 이를 이용한 세포외 소포체의 분리 방법. Applicant: (주)인엑소플랫. The sequence listing filed with the application follows.

SEQUENCE LISTING (19 sequences)

SEQ ID NO: 1 - protein, 238 aa, Homo sapiens
MAVEGGMKCVKFLLYVLLLAFCACAVGLIAVGVGAQLVLSQTIIQGATPGSLLPVVIIAVGVFLFLVAFVGCCGACKENYCLMITFAIFLSLIMLVEVAAAIAGYVFRDKVMSEFNNNFRQQMENYPKNNHTASILDRMQADFKCCGAANYTDWEKIPSMSKNRVPDSCCINVTVGCGINFNEKAIHKEGCVEKIGGWLRKNVLVVAAAALGIAFVEVLGIVFACCLVKSIRSGYEVM

SEQ ID NO: 2 - protein, 236 aa, Homo sapiens
MGVEGCTKCIKYLLFVFNFVFWLAGGVILGVALWLRHDPQTTNLLYLELGDKPAPNTFYVGIYILIAVGAVMMFVGFLGCYGAIQESQCLLGTFFTCLVILFACEVAAGIWGFVNKDQIAKDVKQFYDQALQQAVVDDDANNAKAVVKTFHETLDCCGSSTLTALTTSVLKNNLCPSGSNIISNLFKEDCHQKIDDLFSGKLYLIGIAAIVVAVIMIFEMILSMVLCCGIRNSSVY

SEQ ID NO: 3 - protein, 228 aa, Homo sapiens
MPVKGGTKCIKYLLFGFNFIFWLAGIAVLAIGLWLRFDSQTKSIFEQETNNNNSSFYTGVYILIGAGALMMLVGFLGCCGAVQESQCMLGLFFGFLLVIFAIEIAAAIWGYSHKDEVIKEVQEFYKDTYNKLKTKDEPQRETLKAIHYALNCCGLAGGVEQFISDICPKKDVLETFTVKSCPDAIKEVFDNKFHIIGAVGIGIAVVMIFGMIFSMILCCAIRRNREMV

SEQ ID NO: 4 - protein, 232 aa, Homo sapiens
EPKSCDKTHTCPPCPAPELLGGPSVFLFPPKPKDTLMISRTPEVTCVVVDVSHEDPEVKFNWYVDGVEVHNAKTKPREEQYNSTYRVVSVLTVLHQDWLNGKEYKCKVSNKALPAPIEKTISKAKGQPREPQVYTLPPSRDELTKNQVSLTCLVKGFYPSDIAVEWESNGQPENNYKTTPPVLDSDGSFFLYSKLTVDKSRWQQGNVFSCSVMHEALHNHYTQKSLSLSPGK

SEQ ID NO: 5 - protein, 232 aa, synthetic construct
  REGION 1..232: note = mutated Fc region
EPKSCDKTHTCPPCPAPPLLGGPSVFLFPPKPKDTLMISRTPEVTCVVVDVSHEDPEVKFNWYVDGVEVHNAKTKPREEQYNSTYRVVSVLTVLHQDWLNGKEYKCKVSNKALPAPIEKTISKAKGQPREPQVYTLPPSRDELTKNQVSLTCLVKGFYPSDIAVEWESNGQPENNYKTTPPVLDSDGSFFLYSKLTVDKSRWQQGNVFSCSVMHEALHNHYTQKSLSLSPGK

SEQ ID NO: 6 - protein, 232 aa, synthetic construct; identical to SEQ ID NO: 5
  REGION 1..232: note = mutated CH2 region

SEQ ID NO: 7 - protein, 107 aa, synthetic construct
  REGION 1..107: note = Fc_CH3 region
GQPREPQVYTLPPSRDELTKNQVSLTCLVKGFYPSDIAVEWESNGQPENNYKTTPPVLDSDGSFFLYSKLTVDKSRWQQGNVFSCSVMHEALHNHYTQKSLSLSPGK

SEQ ID NO: 8 - RNA, 23 nt, synthetic construct
  modified_base 3: mod_base = OTHER; note = thymine
  modified_base 7: mod_base = OTHER; note = thymine
  modified_base 15: mod_base = OTHER; note = thymine
  modified_base 18: mod_base = OTHER; note = thymine
  misc_feature 1..23: note = guide RNA
  source 1..23: mol_type = other RNA
cctgagtcagaccataatccagg

SEQ ID NO: 9 - DNA, 800 bp, synthetic construct
  misc_feature 1..800: note = Donor DNA_Left homology arm
  source 1..800: mol_type = other DNA
tgggtgtgcagcaacccctacccccatccctcctggcccttcctgtctggtgacccaaccacttgtgatatggggcagtggggcaaccagccaaccgcctgatgctatcgccatggggcttcccttcgctctcccttctcccctctctccctccccaaccctctcatccctgtccagcccctctccccctttccctcctcccagcgcttgggggtgaggaagggctctgcccacttcaatttgctcctgccctgggctcctggcttgagaggctactgtttgtctagggagggacacatcactcttgctcccttttcctcttcccttctcctggcctaactggccagaggaaccttagtcacagctgatgcgcgcgtgggatgtgcactggaggatagtgagggggcagttctgggagagaattgagctgggagccctggaggcctgtagaaagcattattctaggtcagaaatacgtgtcttgaggtcaaggctttctgggaggtttttgaatttggtcatgtccctgattaaagagccgggaggggatcaggggaggtaggggcaggcaaggatgggtcatccccctaccccacagccaaagaaattccctagaggtgtgagaatctctcttccggatggggtcaagtctgtgtcctaggtgtaccccctgccctccaccatggagggccactgtgttgtggatatggcctaatcctcacctgattttctcttaggcctgtgcagtgggactgattgccgtgggtgtcggggcacagcttgtcctgagtcagaccata

SEQ ID NO: 10 - DNA, 696 bp, synthetic construct
  misc_feature 1..696: note = Donor DNA_Fc region
  source 1..696: mol_type = other DNA
gagcccaagtcctgcgacaagacccacacctgccccccctgccccgcccccccactcctcggcggcccctccgtcttcctcttcccccccaagcccaaggacaccctcatgatctcccgcacccccgaggtcacctgcgtcgtcgtcgacgtctcccacgaggaccccgaggtcaagttcaactggtacgtcgacggcgtcgaggtccacaacgccaagaccaagccccgcgaggagcagtacaactccacctaccgcgtcgtctccgtcctcaccgtcctccaccaggactggctcaacggcaaggagtacaagtgcaaggtctccaacaaggccctccccgcccccatcgagaagaccatctccaaggccaagggccagccccgcgagccccaggtctacaccctccccccctcccgcgacgagctcaccaagaaccaggtctccctcacctgcctcgtcaagggcttctacccctccgacatcgccgtcgagtgggagtccaacggccagcccgagaacaactacaagaccaccccccccgtcctcgactccgacggctccttcttcctctactccaagctcaccgtcgacaagtcccgctggcagcagggcaacgtcttctcctgctccgtcatgcacgaggccctccacaaccactacacccagaagtccctctccctctcccccggcaag

SEQ ID NO: 11 - DNA, 800 bp, synthetic construct
  misc_feature 1..800: note = Donor DNA_Right homology arm
  source 1..800: mol_type = other DNA
atccaaggagctacccctggctctctgttgccagtggtcatcatcgcagtgggtgtcttcctcttcctggtggcttttgtgggctgctgcggggcctgcaaggagaactattgtcttatgatcacggtgagttgggggcgggaccaacatgggcggtctgggactgccagagcagcttggttcgggctcaggaaggtgggtgaggtgggtgggtgaggaagacctttgtgagtgtccagggaccggctgtgccaaaacgggcccctgtaatgcatagactccaaacttgacttctgtcctttgctcctgcagtttgccatctttctgtctcttatcatgttggtggaggtggccgcagccattgctggctatgtgtttagagataaggtaagcagggaataatgggaagggcctgcctcagccgggtctgggaccctggtgcttgaattctgactgcaacagtgctcctccgtactctcaggtgatgtcagagtttaataacaacttccggcagcagatggagaattacccgaaaaacaaccacactgcttcgatcctggacaggatgcaggcagatgtgagtggggttgctgggagcaggggtggtgggaatagagaattctcatctccaaggctgggtgtggtgactcacgcctgtaatctcagcacttttgaaggccgaggtgggcagatcacctgaggtcagaagttcaagactagcctggccaacgtggtgaaaccctgtctctactaaaaatacaaaaattagccaggtgtggtggtgagtgcctgtaatccca

SEQ ID NO: 12 - DNA, 19 bp, synthetic construct
  misc_feature 1..19: note = hCD63(Back)_Forward primer
  source 1..19: mol_type = other DNA
aacaactacaagaccaccc

SEQ ID NO: 13 - DNA, 21 bp, synthetic construct
  misc_feature 1..21: note = hCD63(Back)_Reverse primer
  source 1..21: mol_type = other DNA
gacaaaagcaccatcagaaac

SEQ ID NO: 14 - DNA, 20 bp, synthetic construct
  misc_feature 1..20: note = hCD63(Full_2)_Forward primer
  source 1..20: mol_type = other DNA
accatagagcccaagtcctg

SEQ ID NO: 15 - DNA, 20 bp, synthetic construct
  misc_feature 1..20: note = hCD63(Full_2)_Reverse primer
  source 1..20: mol_type = other DNA
tgaccactggcaacagagag

SEQ ID NO: 16 - DNA, 19 bp, synthetic construct
  misc_feature 1..19: note = hCD63(Front_2)_Forward primer
  source 1..19: mol_type = other DNA
aggggatcaggggaggtag

SEQ ID NO: 17 - DNA, 20 bp, synthetic construct
  misc_feature 1..20: note = hCD63(Front_2)_Reverse primer
  source 1..20: mol_type = other DNA
agggagacctggttcttggt

SEQ ID NO: 18 - DNA, 20 bp, synthetic construct
  source 1..20: mol_type = other DNA
tggaggcctgtagaaagcat

SEQ ID NO: 19 - DNA, 20 bp, synthetic construct
  source 1..20: mol_type = other DNA
ccctggacactcacaaaggt